European Patent Specification EP 3 694 994 B1, published June 12, 2024. Title: A NOVEL METHOD FOR SYNTHESIS OF POLYNUCLEOTIDES USING A DIVERSE LIBRARY OF OLIGONUCLEOTIDES. Applicant: Ribbon Biolabs GmbH. The sequence listing filed with the application follows.

SEQUENCE LISTING (104 sequences)

SEQ ID NO: 1 - DNA, 128 bp, Artificial Sequence
  Polynucleotide
tttcttctttcgagtttctatatccgtcgctggtctgaacggaaaaatcatcgcacaatctatgcctaccgttggctgctcatgcgtccttccgacaatcccatgttcgtctcgcatccgtttcctgc

SEQ ID NO: 2 - DNA, 16 bp, Artificial Sequence
  Oligonucleotide
tttcttctttcgagtt

SEQ ID NO: 3 - DNA, 16 bp, Artificial Sequence
  Oligonucleotide
tagaaactcgaaagaa

SEQ ID NO: 4 - DNA, 16 bp, Artificial Sequence
  Oligonucleotide
tctatatccgtcgctg

SEQ ID NO: 5 - DNA, 16 bp, Artificial Sequence
  Oligonucleotide
agaccagcgacggata

SEQ ID NO: 6 - DNA, 16 bp, Artificial Sequence
  Oligonucleotide
gtctgaacggaaaaat

SEQ ID NO: 7 - DNA, 16 bp, Artificial Sequence
  Oligonucleotide
gatgatttttccgttc

SEQ ID NO: 8 - DNA, 16 bp, Artificial Sequence
  Oligonucleotide
catcgcacaatctatg

SEQ ID NO: 9 - DNA, 16 bp, Artificial Sequence
  Oligonucleotide
taggcatagattgtgc

SEQ ID NO: 10 - DNA, 16 bp, Artificial Sequence
  Oligonucleotide
cctaccgttggctgct

SEQ ID NO: 11 - DNA, 16 bp, Artificial Sequence
  Oligonucleotide
catgagcagccaacgg

SEQ ID NO: 12 - DNA, 16 bp, Artificial Sequence
  Oligonucleotide
catgcgtccttccgac

SEQ ID NO: 13 - DNA, 16 bp, Artificial Sequence
  Oligonucleotide
gattgtcggaaggacg

SEQ ID NO: 14 - DNA, 16 bp, Artificial Sequence
  Oligonucleotide
aatcccatgttcgtct

SEQ ID NO: 15 - DNA, 16 bp, Artificial Sequence
  Oligonucleotide
tgcgagacgaacatgg

SEQ ID NO: 16 - DNA, 16 bp, Artificial Sequence
  Oligonucleotide
cgcatccgtttcctgc

SEQ ID NO: 17 - DNA, 16 bp, Artificial Sequence
  Oligonucleotide
gcgtgcaggaaacgga

SEQ ID NO: 18 - DNA, 36 bp, Artificial Sequence
  Polynucleotide
cctaccgttggctgctaatccgtccttccgacaatc

SEQ ID NO: 19 - DNA, 32 bp, Artificial Sequence
  Polynucleotide
ggcaaccgacgattaggcaggaaggctgttag

SEQ ID NO: 20 - DNA, 36 bp, Artificial Sequence
  Polynucleotide
cctaccgttggctgctcatgcgtccttccgacaatc

SEQ ID NO: 21 - DNA, 32 bp, Artificial Sequence
  Polynucleotide
ggcaaccgacgagtacgcaggaaggctgttag

SEQ ID NO: 22 - DNA, 24 bp, Artificial Sequence
  Polynucleotide
gttggctgctaatccgtccttccg

SEQ ID NO: 23 - DNA, 24 bp, Artificial Sequence
  Polynucleotide
cggaaggacgcatgagcagccaac

SEQ ID NO: 24 - DNA, 18 bp, Artificial Sequence
  Polynucleotide
taatacgactcactatag

SEQ ID NO: 25 - DNA, 16 bp, Artificial Sequence
  Oligonucleotide
aagaaagctcaaagat

SEQ ID NO: 26 - DNA, 608 bp, Artificial Sequence
  Polynucleotide
tttcttctttcgagtttctatatccgtcgctggtctgaacggaaaaatcatcgcacaatctatgcctaccgttggctgctcatgcgtccttccgacaatcccatgttcgtctcgcatccgtttcctgcacgcacccccccctgtactttggaaagcggccatcttaacactctcccaactttttaaatgcgtcgaagccctgggcatctggtttccactagcctagtcgggtgttggatacgccgagagttatggtgtagctgtgtgcgcgaaccgacgggtggaaattgctgaccgattttcaaatagttctcaggaagccgatggcagttacggcttgcgactcggggcaccgtgagcctcttctccctctagaagtcgaagcaagggacactatcctaaatgccatggactagcgcgcgcgaaatcgatgcactccttattaatgtgatctgcgcaagttgttcagccatcggtcattttgcgttgatattcggttctttgatttgcgtgccatgcttataacaggacacttattgtgccccagctcttctcatgcaagtgcggttttctctagctactgtggtgtgcgctcatcaatactccag

SEQ ID NO: 27 - DNA, 16 bp, Artificial Sequence
  Oligonucleotide
tttcttctttcgagtt

SEQ ID NO: 28 - DNA, 16 bp, Artificial Sequence
  Oligonucleotide
tagaaactcgaaagaa

SEQ ID NO: 29 - DNA, 16 bp, Artificial Sequence
  Oligonucleotide
tctatatccgtcgctg

SEQ ID NO: 30 - DNA, 16 bp, Artificial Sequence
  Oligonucleotide
agaccagcgacggata

SEQ ID NO: 31 - DNA, 16 bp, Artificial Sequence
  Oligonucleotide
gtctgaacggaaaaat

SEQ ID NO: 32 - DNA, 16 bp, Artificial Sequence
  Oligonucleotide
gatgatttttccgttc

SEQ ID NO: 33 - DNA, 16 bp, Artificial Sequence
  Oligonucleotide
catcgcacaatctatg

SEQ ID NO: 34 - DNA, 16 bp, Artificial Sequence
  Oligonucleotide
taggcatagattgtgc

SEQ ID NO: 35 - DNA, 16 bp, Artificial Sequence
  Oligonucleotide
cctaccgttggctgct

SEQ ID NO: 36 - DNA, 16 bp, Artificial Sequence
  Oligonucleotide
catgagcagccaacgg

SEQ ID NO: 37 - DNA, 16 bp, Artificial Sequence
  Oligonucleotide
catgcgtccttccgac

SEQ ID NO: 38 - DNA, 16 bp, Artificial Sequence
  Oligonucleotide
gattgtcggaaggacg

SEQ ID NO: 39 - DNA, 16 bp, Artificial Sequence
  Oligonucleotide
aatcccatgttcgtct

SEQ ID NO: 40 - DNA, 16 bp, Artificial Sequence
  Oligonucleotide
tgcgagacgaacatgg

SEQ ID NO: 41 - DNA, 16 bp, Artificial Sequence
  Oligonucleotide
cgcatccgtttcctgc

SEQ ID NO: 42 - DNA, 16 bp, Artificial Sequence
  Oligonucleotide
gcgtgcaggaaacgga

SEQ ID NO: 43 - DNA, 16 bp, Artificial Sequence
  Oligonucleotide
acgcacccccccctgt

SEQ ID NO: 44 - DNA, 16 bp, Artificial Sequence
  Oligonucleotide
aagtacaggggggggt

SEQ ID NO: 45 - DNA, 16 bp, Artificial Sequence
  Oligonucleotide
actttggaaagcggcc

SEQ ID NO: 46 - DNA, 16 bp, Artificial Sequence
  Oligonucleotide
agatggccgctttcca

SEQ ID NO: 47 - DNA, 16 bp, Artificial Sequence
  Oligonucleotide
atcttaacactctccc

SEQ ID NO: 48 - DNA, 16 bp, Artificial Sequence
  Oligonucleotide
agttgggagagtgtta

SEQ ID NO: 49 - DNA, 16 bp, Artificial Sequence
  Oligonucleotide
aactttttaaatgcgt

SEQ ID NO: 50 - DNA, 16 bp, Artificial Sequence
  Oligonucleotide
ttcgacgcatttaaaa

SEQ ID NO: 51 - DNA, 16 bp, Artificial Sequence
  Oligonucleotide
cgaagccctgggcatc

SEQ ID NO: 52 - DNA, 16 bp, Artificial Sequence
  Oligonucleotide
accagatgcccagggc

SEQ ID NO: 53 - DNA, 16 bp, Artificial Sequence
  Oligonucleotide
tggtttccactagcct

SEQ ID NO: 54 - DNA, 16 bp, Artificial Sequence
  Oligonucleotide
gactaggctagtggaa

SEQ ID NO: 55 - DNA, 16 bp, Artificial Sequence
  Oligonucleotide
agtcgggtgttggata

SEQ ID NO: 56 - DNA, 16 bp, Artificial Sequence
  Oligonucleotide
ggcgtatccaacaccc

SEQ ID NO: 57 - DNA, 16 bp, Artificial Sequence
  Oligonucleotide
cgccgagagttatggt

SEQ ID NO: 58 - DNA, 16 bp, Artificial Sequence
  Oligonucleotide
ctacaccataactctc

SEQ ID NO: 59 - DNA, 16 bp, Artificial Sequence
  Oligonucleotide
gtagctgtgtgcgcga

SEQ ID NO: 60 - DNA, 16 bp, Artificial Sequence
  Oligonucleotide
cggttcgcgcacacag

SEQ ID NO: 61 - DNA, 16 bp, Artificial Sequence
  Oligonucleotide
accgacgggtggaaat

SEQ ID NO: 62 - DNA, 16 bp, Artificial Sequence
  Oligonucleotide
agcaatttccacccgt

SEQ ID NO: 63 - DNA, 16 bp, Artificial Sequence
  Oligonucleotide
tgctgaccgattttca

SEQ ID NO: 64 - DNA, 16 bp, Artificial Sequence
  Oligonucleotide
tatttgaaaatcggtc

SEQ ID NO: 65 - DNA, 16 bp, Artificial Sequence
  Oligonucleotide
aatagttctcaggaag

SEQ ID NO: 66 - DNA, 16 bp, Artificial Sequence
  Oligonucleotide
tcggcttcctgagaac

SEQ ID NO: 67 - DNA, 16 bp, Artificial Sequence
  Oligonucleotide
ccgatggcagttacgg

SEQ ID NO: 68 - DNA, 16 bp, Artificial Sequence
  Oligonucleotide
caagccgtaactgcca

SEQ ID NO: 69 - DNA, 16 bp, Artificial Sequence
  Oligonucleotide
cttgcgactcggggca

SEQ ID NO: 70 - DNA, 16 bp, Artificial Sequence
  Oligonucleotide
acggtgccccgagtcg

SEQ ID NO: 71 - DNA, 16 bp, Artificial Sequence
  Oligonucleotide
ccgtgagcctcttctc

SEQ ID NO: 72 - DNA, 16 bp, Artificial Sequence
  Oligonucleotide
gagggagaagaggctc

SEQ ID NO: 73 - DNA, 16 bp, Artificial Sequence
  Oligonucleotide
cctctagaagtcgaag

SEQ ID NO: 74 - DNA, 16 bp, Artificial Sequence
  Oligonucleotide
cttgcttcgacttcta

SEQ ID NO: 75 - DNA, 16 bp, Artificial Sequence
  Oligonucleotide
caagggacactatcct

SEQ ID NO: 76 - DNA, 16 bp, Artificial Sequence
  Oligonucleotide
atttaggatagtgtcc

SEQ ID NO: 77 - DNA, 16 bp, Artificial Sequence
  Oligonucleotide
aaatgccatggactag

SEQ ID NO: 78 - DNA, 16 bp, Artificial Sequence
  Oligonucleotide
cgcgctagtccatggc

SEQ ID NO: 79 - DNA, 16 bp, Artificial Sequence
  Oligonucleotide
cgcgcgcgaaatcgat

SEQ ID NO: 80 - DNA, 16 bp, Artificial Sequence
  Oligonucleotide
gtgcatcgatttcgcg

SEQ ID NO: 81 - DNA, 16 bp, Artificial Sequence
  Oligonucleotide
gcactccttattaatg

SEQ ID NO: 82 - DNA, 16 bp, Artificial Sequence
  Oligonucleotide
atcacattaataagga

SEQ ID NO: 83 - DNA, 16 bp, Artificial Sequence
  Oligonucleotide
tgatctgcgcaagttg

SEQ ID NO: 84 - DNA, 16 bp, Artificial Sequence
  Oligonucleotide
tgaacaacttgcgcag

SEQ ID NO: 85 - DNA, 16 bp, Artificial Sequence
  Oligonucleotide
ttcagccatcggtcat

SEQ ID NO: 86 - DNA, 16 bp, Artificial Sequence
  Oligonucleotide
caaaatgaccgatggc

SEQ ID NO: 87 - DNA, 16 bp, Artificial Sequence
  Oligonucleotide
tttgcgttgatattcg

SEQ ID NO: 88 - DNA, 16 bp, Artificial Sequence
  Oligonucleotide
gaaccgaatatcaacg

SEQ ID NO: 89 - DNA, 16 bp, Artificial Sequence
  Oligonucleotide
gttctttgatttgcgt

SEQ ID NO: 90 - DNA, 16 bp, Artificial Sequence
  Oligonucleotide
tggcacgcaaatcaaa

SEQ ID NO: 91 - DNA, 16 bp, Artificial Sequence
  Oligonucleotide
gccatgcttataacag

SEQ ID NO: 92 - DNA, 16 bp, Artificial Sequence
  Oligonucleotide
tgtcctgttataagca

SEQ ID NO: 93 - DNA, 16 bp, Artificial Sequence
  Oligonucleotide
gacacttattgtgccc

SEQ ID NO: 94 - DNA, 16 bp, Artificial Sequence
  Oligonucleotide
gctggggcacaataag

SEQ ID NO: 95 - DNA, 16 bp, Artificial Sequence
  Oligonucleotide
cagctcttctcatgca

SEQ ID NO: 96 - DNA, 16 bp, Artificial Sequence
  Oligonucleotide
cacttgcatgagaaga

SEQ ID NO: 97 - DNA, 16 bp, Artificial Sequence
  Oligonucleotide
agtgcggttttctcta

SEQ ID NO: 98 - DNA, 16 bp, Artificial Sequence
  Oligonucleotide
tagctagagaaaaccg

SEQ ID NO: 99 - DNA, 16 bp, Artificial Sequence
  Oligonucleotide
gctactgtggtgtgcg

SEQ ID NO: 100 - DNA, 16 bp, Artificial Sequence
  Oligonucleotide
tgagcgcacaccacag

SEQ ID NO: 101 - DNA, 16 bp, Artificial Sequence
  Oligonucleotide
ctcatcaatactccag

SEQ ID NO: 102 - DNA, 16 bp, Artificial Sequence
  Oligonucleotide
ttatctggagtattga

SEQ ID NO: 103 - DNA, 32 bp, Artificial Sequence
  Primer
tttcttctttcgagtttctatatccgtcgctg

SEQ ID NO: 104 - DNA, 25 bp, Artificial Sequence
  Primer
ttatctggagtattgatgagcgcac